European Patent Application EP 4 763 987 A2, published June 24, 2026. Title: VARIANT RNAi AGAINST ALPHA-SYNUCLEIN. Applicant: Genzyme Corporation. Application EP. The sequence listing filed with the application follows.

SEQUENCE LISTING (70 sequences)

SEQ ID NO: 1 - RNA, 21 nt, synthetic construct
  misc_feature 1..21: note = Synthetic Construct
  source 1..21: mol_type = other RNA
catcggaactgagcacttgta

SEQ ID NO: 2 - RNA, 22 nt, synthetic construct
  misc_feature 1..22: note = Synthetic Construct
  source 1..22: mol_type = other RNA
aggttcgtagtcttgataccct

SEQ ID NO: 3 - RNA, 22 nt, synthetic construct
  misc_feature 1..22: note = Synthetic Construct
  source 1..22: mol_type = other RNA
ttaaccgccactttctaacctt

SEQ ID NO: 4 - RNA, 21 nt, synthetic construct
  misc_feature 1..21: note = Synthetic Construct
  source 1..21: mol_type = other RNA
acgttggaactgagcacttgt

SEQ ID NO: 5 - RNA, 21 nt, synthetic construct
  misc_feature 1..21: note = Synthetic Construct
  source 1..21: mol_type = other RNA
ttccaacatttgtcacttgct

SEQ ID NO: 6 - RNA, 21 nt, synthetic construct
  misc_feature 1..21: note = Synthetic Construct
  source 1..21: mol_type = other RNA
tcgtccaacatttgtcacttg

SEQ ID NO: 7 - RNA, 21 nt, synthetic construct
  misc_feature 1..21: note = Synthetic Construct
  source 1..21: mol_type = other RNA
tgggcgcattggaactgagca

SEQ ID NO: 8 - RNA, 21 nt, synthetic construct
  misc_feature 1..21: note = Synthetic Construct
  source 1..21: mol_type = other RNA
tgggcacattggaactgagca

SEQ ID NO: 9 - RNA, 21 nt, synthetic construct
  misc_feature 1..21: note = Synthetic Construct
  source 1..21: mol_type = other RNA
gtcgtcgaatggccactccca

SEQ ID NO: 10 - RNA, 22 nt, synthetic construct
  misc_feature 1..22: note = Synthetic Construct
  source 1..22: mol_type = other RNA
ggttcgtagtcttgataccctt

SEQ ID NO: 11 - RNA, 21 nt, synthetic construct
  misc_feature 1..21: note = Synthetic Construct
  source 1..21: mol_type = other RNA
tagcagcagccacaactccct

SEQ ID NO: 12 - RNA, 21 nt, synthetic construct
  misc_feature 1..21: note = Synthetic Construct
  source 1..21: mol_type = other RNA
ttcgaacatttgtcacttgct

SEQ ID NO: 13 - RNA, 21 nt, synthetic construct
  misc_feature 1..21: note = Synthetic Construct
  source 1..21: mol_type = other RNA
tagccgccacaactccctcct

SEQ ID NO: 14 - RNA, 21 nt, synthetic construct
  misc_feature 1..21: note = Synthetic Construct
  source 1..21: mol_type = other RNA
tgcgctttggtcttctcagcc

SEQ ID NO: 15 - RNA, 21 nt, synthetic construct
  misc_feature 1..21: note = Synthetic Construct
  source 1..21: mol_type = other RNA
tagccgcagccacaactccct

SEQ ID NO: 16 - RNA, 21 nt, synthetic construct
  misc_feature 1..21: note = Synthetic Construct
  source 1..21: mol_type = other RNA
tagcagccacaactccctcct

SEQ ID NO: 17 - RNA, 21 nt, synthetic construct
  misc_feature 1..21: note = Synthetic Construct
  source 1..21: mol_type = other RNA
tcggcacattggaactgagca

SEQ ID NO: 18 - RNA, 21 nt, synthetic construct
  misc_feature 1..21: note = Synthetic Construct
  source 1..21: mol_type = other RNA
atgacggggcacattggaact

SEQ ID NO: 19 - RNA, 21 nt, synthetic construct
  misc_feature 1..21: note = Synthetic Construct
  source 1..21: mol_type = other RNA
atgactgggcacattggaact

SEQ ID NO: 20 - RNA, 21 nt, synthetic construct
  misc_feature 1..21: note = Synthetic Construct
  source 1..21: mol_type = other RNA
taagtcgtagtcacttaggtg

SEQ ID NO: 21 - RNA, 21 nt, synthetic construct
  misc_feature 1..21: note = Synthetic Construct
  source 1..21: mol_type = other RNA
ctccgcagcagccacaactcc

SEQ ID NO: 22 - RNA, 21 nt, synthetic construct
  misc_feature 1..21: note = Synthetic Construct
  source 1..21: mol_type = other RNA
tcatgactgggcacattggaa

SEQ ID NO: 23 - RNA, 21 nt, synthetic construct
  misc_feature 1..21: note = Synthetic Construct
  source 1..21: mol_type = other RNA
aaatacgtggtagtcacttag

SEQ ID NO: 24 - RNA, 21 nt, synthetic construct
  misc_feature 1..21: note = Synthetic Construct
  source 1..21: mol_type = other RNA
tgctctttggtcttctcagcc

SEQ ID NO: 25 - RNA, 21 nt, synthetic construct
  misc_feature 1..21: note = Synthetic Construct
  source 1..21: mol_type = other RNA
aacgtttgtcacttgctcttt

SEQ ID NO: 26 - RNA, 21 nt, synthetic construct
  misc_feature 1..21: note = Synthetic Construct
  source 1..21: mol_type = other RNA
aaataagtggtagtcacttag

SEQ ID NO: 27 - RNA, 21 nt, synthetic construct
  misc_feature 1..21: note = Synthetic Construct
  source 1..21: mol_type = other RNA
ttagaaataagtggtagtcac

SEQ ID NO: 28 - RNA, 21 nt, synthetic construct
  misc_feature 1..21: note = Synthetic Construct
  source 1..21: mol_type = other RNA
aatacgtggtagtcacttagg

SEQ ID NO: 29 - RNA, 21 nt, synthetic construct
  misc_feature 1..21: note = Synthetic Construct
  source 1..21: mol_type = other RNA
actgcgcacattggaactgag

SEQ ID NO: 30 - RNA, 19 nt, synthetic construct
  misc_feature 1..19: note = Synthetic Construct
  source 1..19: mol_type = other RNA
tacaagtgcagttccgatg

SEQ ID NO: 31 - RNA, 20 nt, synthetic construct
  misc_feature 1..20: note = Synthetic Construct
  source 1..20: mol_type = other RNA
aaggttagaatggcggttaa

SEQ ID NO: 32 - RNA, 20 nt, synthetic construct
  misc_feature 1..20: note = Synthetic Construct
  source 1..20: mol_type = other RNA
aaggttagaatggcggttaa

SEQ ID NO: 33 - RNA, 19 nt, synthetic construct
  misc_feature 1..19: note = Synthetic Construct
  source 1..19: mol_type = other RNA
acaagtgcagttccaacgt

SEQ ID NO: 34 - RNA, 19 nt, synthetic construct
  misc_feature 1..19: note = Synthetic Construct
  source 1..19: mol_type = other RNA
agcaagtgaaatgttggaa

SEQ ID NO: 35 - RNA, 19 nt, synthetic construct
  misc_feature 1..19: note = Synthetic Construct
  source 1..19: mol_type = other RNA
caagtgacatgttggacga

SEQ ID NO: 36 - RNA, 19 nt, synthetic construct
  misc_feature 1..19: note = Synthetic Construct
  source 1..19: mol_type = other RNA
tgctcagtcaatgcgccta

SEQ ID NO: 37 - RNA, 19 nt, synthetic construct
  misc_feature 1..19: note = Synthetic Construct
  source 1..19: mol_type = other RNA
tgctcagtcaatgtgccta

SEQ ID NO: 38 - RNA, 19 nt, synthetic construct
  misc_feature 1..19: note = Synthetic Construct
  source 1..19: mol_type = other RNA
tgggagtgcattcgacgat

SEQ ID NO: 39 - RNA, 20 nt, synthetic construct
  misc_feature 1..20: note = Synthetic Construct
  source 1..20: mol_type = other RNA
aagggtatcaactacgaacc

SEQ ID NO: 40 - RNA, 19 nt, synthetic construct
  misc_feature 1..19: note = Synthetic Construct
  source 1..19: mol_type = other RNA
agggagttggctgctgcta

SEQ ID NO: 41 - RNA, 19 nt, synthetic construct
  misc_feature 1..19: note = Synthetic Construct
  source 1..19: mol_type = other RNA
agcaagtgaaatgttcgaa

SEQ ID NO: 42 - RNA, 19 nt, synthetic construct
  misc_feature 1..19: note = Synthetic Construct
  source 1..19: mol_type = other RNA
aggagggatgtggcggcta

SEQ ID NO: 43 - RNA, 19 nt, synthetic construct
  misc_feature 1..19: note = Synthetic Construct
  source 1..19: mol_type = other RNA
ggctgagaaccaaagcgta

SEQ ID NO: 44 - RNA, 19 nt, synthetic construct
  misc_feature 1..19: note = Synthetic Construct
  source 1..19: mol_type = other RNA
agggagttggctgcggcta

SEQ ID NO: 45 - RNA, 19 nt, synthetic construct
  misc_feature 1..19: note = Synthetic Construct
  source 1..19: mol_type = other RNA
aggagggatgtggctgcta

SEQ ID NO: 46 - RNA, 19 nt, synthetic construct
  misc_feature 1..19: note = Synthetic Construct
  source 1..19: mol_type = other RNA
tgctcagtcaatgtgccga

SEQ ID NO: 47 - RNA, 19 nt, synthetic construct
  misc_feature 1..19: note = Synthetic Construct
  source 1..19: mol_type = other RNA
agttccaatgccccgtcat

SEQ ID NO: 48 - RNA, 19 nt, synthetic construct
  misc_feature 1..19: note = Synthetic Construct
  source 1..19: mol_type = other RNA
agttccaatgcccagtcat

SEQ ID NO: 49 - RNA, 19 nt, synthetic construct
  misc_feature 1..19: note = Synthetic Construct
  source 1..19: mol_type = other RNA
cacctaagactacgactta

SEQ ID NO: 50 - RNA, 19 nt, synthetic construct
  misc_feature 1..19: note = Synthetic Construct
  source 1..19: mol_type = other RNA
ggagttgtctgctgcggag

SEQ ID NO: 51 - RNA, 19 nt, synthetic construct
  misc_feature 1..19: note = Synthetic Construct
  source 1..19: mol_type = other RNA
ttccaatgcccagtcatga

SEQ ID NO: 52 - RNA, 19 nt, synthetic construct
  misc_feature 1..19: note = Synthetic Construct
  source 1..19: mol_type = other RNA
ctaagtgaaccacgtattt

SEQ ID NO: 53 - RNA, 19 nt, synthetic construct
  misc_feature 1..19: note = Synthetic Construct
  source 1..19: mol_type = other RNA
ggctgagaaccaaagagta

SEQ ID NO: 54 - RNA, 19 nt, synthetic construct
  misc_feature 1..19: note = Synthetic Construct
  source 1..19: mol_type = other RNA
aaagagcatgacaaacgtt

SEQ ID NO: 55 - RNA, 19 nt, synthetic construct
  misc_feature 1..19: note = Synthetic Construct
  source 1..19: mol_type = other RNA
ctaagtgaaccacttattt

SEQ ID NO: 56 - RNA, 19 nt, synthetic construct
  misc_feature 1..19: note = Synthetic Construct
  source 1..19: mol_type = other RNA
gtgactaccttatttctaa

SEQ ID NO: 57 - RNA, 19 nt, synthetic construct
  misc_feature 1..19: note = Synthetic Construct
  source 1..19: mol_type = other RNA
cctaagtgtaccacgtatt

SEQ ID NO: 58 - RNA, 19 nt, synthetic construct
  misc_feature 1..19: note = Synthetic Construct
  source 1..19: mol_type = other RNA
ctcagttcatgtgcgcagt

SEQ ID NO: 59 - DNA, 19 bp, synthetic construct
  misc_feature 1..19: note = Synthetic Construct
  source 1..19: mol_type = other DNA
gttttggccactgactgac

SEQ ID NO: 60 - RNA, 19 nt, synthetic construct
  misc_feature 1..19: note = Synthetic Construct
  source 1..19: mol_type = other RNA
gttttggccactgactgac

SEQ ID NO: 61 - RNA, 59 nt, synthetic construct
  misc_feature 1..59: note = Synthetic Construct
  source 1..59: mol_type = other RNA
tgctctttggtcttctcagccgttttggccactgactgacggctgagaaccaaagagta

SEQ ID NO: 62 - DNA, 59 bp, synthetic construct
  misc_feature 1..59: note = Synthetic Construct
  source 1..59: mol_type = other DNA
tgctctttggtcttctcagccgttttggccactgactgacggctgagaaccaaagagta

SEQ ID NO: 63 - RNA, 59 nt, synthetic construct
  misc_feature 1..59: note = Synthetic Construct
  source 1..59: mol_type = other RNA
tgggcacattggaactgagcagttttggccactgactgactgctcagtcaatgtgccta

SEQ ID NO: 64 - DNA, 59 bp, synthetic construct
  misc_feature 1..59: note = Synthetic Construct
  source 1..59: mol_type = other DNA
tgggcacattggaactgagcagttttggccactgactgactgctcagtcaatgtgccta

SEQ ID NO: 65 - DNA, 3455 bp, synthetic construct
  misc_feature 1..3455: note = Synthetic Construct
  source 1..3455: mol_type = other DNA
ttggccactccctctctgcgcgctcgctcgctcactgaggccgcccgggcaaagcccgggcgtcgggcgacctttggtcgcccggcctcagtgagcgagcgagcgcgcagagagggagtggccaactccatcactaggggttccttacgtacaattgggatcccggaccgtcgacattgattattgactagttattaatagtaatcaattacggggtcattagttcatagcccatatatggagttccgcgttacataacttacggtaaatggcccgcctggctgaccgcccaacgacccccgcccattgacgtcaataatgacgtatgttcccatagtaacgccaatagggactttccattgacgtcaatgggtggagtatttacggtaaactgcccacttggcagtacatcaagtgtatcatatgccaagtacgccccctattgacgtcaatgacggtaaatggcccgcctggcattatgcccagtacatgaccttatgggactttcctacttggcagtacatctacgtattagtcatcgctattaccatggtcgaggtgagccccacgttctgcttcactctccccatctcccccccctccccacccccaattttgtatttatttattttttaattattttgtgcagcgatgggggcggggggggggggggggcgcgcgccaggcggggcggggcggggcgaggggcggggcggggcgaggcggagaggtgcggcggcagccaatcagagcggcgcgctccgaaagtttccttttatggcgaggcggcggcggcggcggccctataaaaagcgaagcgcgcggcgggcggggagtcgctgcgacgctgccttcgccccgtgccccgctccgccgccgcctcgcgccgcccgccccggctctgactgaccgcgttactcccacaggtgagcgggcgggacggcccttctcctccgggctgtaattagcgcttggtttaatgacggcttgtttcttttctgtggctgcgtgaaagccttgaggggctccgggagggccctttgtgcggggggagcggctcggggggtgcgtgcgtgtgtgtgtgcgtggggagcgccgcgtgcggctccgcgctgcccggcggctgtgagcgctgcgggcgcggcgcggggctttgtgcgctccgcagtgtgcgcgaggggagcgcggccgggggcggtgccccgcggtgcggggggggctgcgaggggaacaaaggctgcgtgcggggtgtgtgcgtgggggggtgagcagggggtgtgggcgcgtcggtcgggctgcaaccccccctgcacccccctccccgagttgctgagcacggcccggcttcgggtgcggggctccgtacggggcgtggcgcggggctcgccgtgccgggcggggggtggcggcaggtgggggtgccgggcggggcggggccgcctcgggccggggagggctcgggggaggggcgcggcggcccccggagcgccggcggctgtcgaggcgcggcgagccgcagccattgccttttatggtaatcgtgcgagagggcgcagggacttcctttgtcccaaatctgtgcggagccgaaatctgggaggcgccgccgcaccccctctagcgggcgcggggcgaagcggtgcggcgccggcaggaaggaaatgggcggggagggccttcgtgcgtcgccgcgccgccgtccccttctccctctccagcctcggggctgtccgcggggggacggctgccttcgggggggacggggcagggcggggttcggcttctggcgtgtgaccggcggctctagagcctctgctaaccatgttcatgccttcttctttttcctacagctcctgggcaacgtgctggttattgtgctgtctcatcattttggcaaagaattcttcgaaagatctgctagcctagactggaggcttgctgaaggctgtatgctgtgctctttggtcttctcagccgttttggccactgactgacggctgagaaccaaagagtacaggacacaaggcctgttactagcactcacatggaacaaatggcccagatctggccgcactcgagatatcgagctcgctgatcagcctcgactgtgccttctagttgccagccatctgttgtttgcccctcccccgtgccttccttgaccctggaaggtgccactcccactgtcctttcctaataaaatgaggaaattgcatcgcattgtctgagtaggtgtcattctattctggggggtggggtggggcaggacagcaagggggaggattgggaagacaatagcaggcatgctggggagctagagtcgaccggaccggtggaagtcctcttcctcggtgtccttgacttcaaagggtctctcccatttgcctggagagaggggaaggtgggcatcaccaggggtgagtgaaggtttggaagagtgtagcagaataagaaaccatgagtcccctccctgagaagccctgagcccccttgacgacacacatccctcgaggctcagcttcatcatctgtaaaaggtgctgaaactgaccatccaagctgccgaaaaagattgtgtggggataattcaaaactagaggaagatgcagaatttctacatcgtggcgatgtcaggctaagagatgccatcgtggctgtgcatttttattggaatcatatgtttatttgagggtgtcttggatattacaaataaaatgttggagcatcaggcatatttggtaccttctgtctaaggctccctgccccttgttaattggcagctcagttattcatccagggcaaacattctgcttactattcctgagagctttcctcatcctctagattggcaggggaaatgcagatgcctgagcagcctcccctctgccataccaacagagcttcaccatcgaggcatgcagagtggacaggggcctcagggacccctgatcccagctttctcattggacagaaggaggagactggggctggagagggacctgggcccccactaaggccacagcagagccaggactttagctgtgctgactgcagcctggcttgcctccactgccctcctttgcctcaagagcaagggagcctcagagtggaggaagcagcccctggccttgcctcccacctcccctcccctatgctgttttcctgggacagtgggagctggcttagaatgccctggggcccccaggaccctggcattttaacccctcaggggcaggaaggcagcctgagatacagaagagtccatcacctgctgtatgccacacaccatccccacagtcgacatttaaattaggaacccctagtgatggagttggccactccctctctgcgcgctcgctcgctcactgaggccgcccgggcaaagcccgggcgtcgggcgacctttggtcgcccggcctcagtgagcgagcgagcgcgcagagagggagtggccaa

SEQ ID NO: 66 - DNA, 1091 bp, synthetic construct
  misc_feature 1..1091: note = Synthetic Construct
  source 1..1091: mol_type = other DNA
attgtctgagtaggtgtcattctattctggggggtggggtggggcaggacagcaagggggaggattgggaagacaatagcaggcatgctggggagctagagtcgaccggaccggtggaagtcctcttcctcggtgtccttgacttcaaagggtctctcccatttgcctggagagaggggaaggtgggcatcaccaggggtgagtgaaggtttggaagagtgtagcagaataagaaaccatgagtcccctccctgagaagccctgagcccccttgacgacacacatccctcgaggctcagcttcatcatctgtaaaaggtgctgaaactgaccatccaagctgccgaaaaagattgtgtggggataattcaaaactagaggaagatgcagaatttctacatcgtggcgatgtcaggctaagagatgccatcgtggctgtgcatttttattggaatcatatgtttatttgagggtgtcttggatattacaaataaaatgttggagcatcaggcatatttggtaccttctgtctaaggctccctgccccttgttaattggcagctcagttattcatccagggcaaacattctgcttactattcctgagagctttcctcatcctctagattggcaggggaaatgcagatgcctgagcagcctcccctctgccataccaacagagcttcaccatcgaggcatgcagagtggacaggggcctcagggacccctgatcccagctttctcattggacagaaggaggagactggggctggagagggacctgggcccccactaaggccacagcagagccaggactttagctgtgctgactgcagcctggcttgcctccactgccctcctttgcctcaagagcaagggagcctcagagtggaggaagcagcccctggccttgcctcccacctcccctcccctatgctgttttcctgggacagtgggagctggcttagaatgccctggggcccccaggaccctggcattttaacccctcaggggcaggaaggcagcctgagatacagaagagtccatcacctgctgtatgccacacaccatccccacagtcgacatttaaatt

SEQ ID NO: 67 - DNA, 72 bp, synthetic construct
  misc_feature 1..72: note = Synthetic Construct
  source 1..72: mol_type = other DNA
ctggaggcttgctgaaggctgtatgctgcaggacacaaggcctgttactagcactcacatggaacaaatggc

SEQ ID NO: 68 - DNA, 128 bp, synthetic construct
  misc_feature 1..128: note = Synthetic Construct
  source 1..128: mol_type = other DNA
ctggaggcttgctgaaggctgtatgctgtacgatctaatatcgctcgttttggccactgactgacgagcgatatgatcgtacgacaggacacaaggcctgttactagcactcacatggaacaaatggc

SEQ ID NO: 69 - DNA, 78 bp, synthetic construct
  misc_feature 1..78: note = Synthetic Construct
  source 1..78: mol_type = other DNA
cactccctctctgcgcgctcgctcgctcactgaggccgggcgaccaaaggtcgcccacgcccgggctttgcccgggcg

SEQ ID NO: 70 - DNA, 145 bp, synthetic construct
  misc_feature 1..145: note = Synthetic Construct
  source 1..145: mol_type = other DNA
ttggccactccctctctgcgcgctcgctcgctcactgaggccgcccgggcaaagcccgggcgtcgggcgacctttggtcgcccggcctcagtgagcgagcgagcgcgcagagagggagtggccaactccatcactaggggttcct